European Patent Application EP 4 520 349 A1, published March 12, 2025. Title: Interfering RNA for inhibiting b7-h3 gene expression and use thereof. Applicant: JENKEM TECHNOLOGY CO., LTD. (BEIJING). Application WO PCT/CN2023/104455, filed June 30, 2023. The sequence listing filed with the application follows.

SEQUENCE LISTING (91 sequences)

SEQ ID NO: 1 - DNA, 19 bp, synthetic construct
  source 1..19: mol_type = other DNA
caacgagcagggcttgttt

SEQ ID NO: 2 - DNA, 19 bp, synthetic construct
  source 1..19: mol_type = other DNA
gtctgtctgtctcattgca

SEQ ID NO: 3 - DNA, 19 bp, synthetic construct
  source 1..19: mol_type = other DNA
gctggagaaagatcaaaca

SEQ ID NO: 4 - DNA, 19 bp, synthetic construct
  source 1..19: mol_type = other DNA
gcagctgacagacaccaaa

SEQ ID NO: 5 - DNA, 19 bp, synthetic construct
  source 1..19: mol_type = other DNA
ggtgcacagtttcaccgaa

SEQ ID NO: 6 - DNA, 19 bp, synthetic construct
  source 1..19: mol_type = other DNA
agaccactgtgcagcctta

SEQ ID NO: 7 - DNA, 19 bp, synthetic construct
  source 1..19: mol_type = other DNA
agatgtcagcactgtgtta

SEQ ID NO: 8 - DNA, 19 bp, synthetic construct
  source 1..19: mol_type = other DNA
gctttcgtgtgctggagaa

SEQ ID NO: 9 - DNA, 19 bp, synthetic construct
  source 1..19: mol_type = other DNA
agaagatgatggacaagaa

SEQ ID NO: 10 - DNA, 19 bp, synthetic construct
  source 1..19: mol_type = other DNA
agatgatggacaagaaata

SEQ ID NO: 11 - DNA, 19 bp, synthetic construct
  source 1..19: mol_type = other DNA
caatggacatgattcccaa

SEQ ID NO: 12 - DNA, 19 bp, synthetic construct
  source 1..19: mol_type = other DNA
ggacatgattcccaagtca

SEQ ID NO: 13 - DNA, 19 bp, synthetic construct
  source 1..19: mol_type = other DNA
ccttagttctctaagtcat

SEQ ID NO: 14 - DNA, 19 bp, synthetic construct
  source 1..19: mol_type = other DNA
gatgcaatattcagactga

SEQ ID NO: 15 - DNA, 19 bp, synthetic construct
  source 1..19: mol_type = other DNA
ccttcctcctcttgctcta

SEQ ID NO: 16 - DNA, 19 bp, synthetic construct
  source 1..19: mol_type = other DNA
ccattcagttgatgtttat

SEQ ID NO: 17 - DNA, 19 bp, synthetic construct
  source 1..19: mol_type = other DNA
gttgatgtttattgagcaa

SEQ ID NO: 18 - DNA, 19 bp, synthetic construct
  source 1..19: mol_type = other DNA
gatgtttattgagcaacta

SEQ ID NO: 19 - DNA, 19 bp, synthetic construct
  source 1..19: mol_type = other DNA
gataaagttcctccctcaa

SEQ ID NO: 20 - DNA, 19 bp, synthetic construct
  source 1..19: mol_type = other DNA
gctgggagacagacaacta

SEQ ID NO: 21 - DNA, 19 bp, synthetic construct
  source 1..19: mol_type = other DNA
ggagacagacaactaacta

SEQ ID NO: 22 - DNA, 19 bp, synthetic construct
  source 1..19: mol_type = other DNA
agacagacaactaactaca

SEQ ID NO: 23 - DNA, 19 bp, synthetic construct
  source 1..19: mol_type = other DNA
gctcaaggcttcctggata

SEQ ID NO: 24 - DNA, 19 bp, synthetic construct
  source 1..19: mol_type = other DNA
ggtagagtgagacttcaga

SEQ ID NO: 25 - DNA, 19 bp, synthetic construct
  source 1..19: mol_type = other DNA
gtgaggacttctaatttaa

SEQ ID NO: 26 - RNA, 21 nt, synthetic construct
  source 1..21: mol_type = other RNA
  modified_base 20..21: mod_base = OTHER; note = Thymine
caacgagcagggcttgttttt

SEQ ID NO: 27 - RNA, 21 nt, synthetic construct
  source 1..21: mol_type = other RNA
  modified_base 20..21: mod_base = OTHER; note = Thymine
aaacaagccctgctcgttgtt

SEQ ID NO: 28 - RNA, 21 nt, synthetic construct
  source 1..21: mol_type = other RNA
  modified_base 20..21: mod_base = OTHER; note = Thymine
gtctgtctgtctcattgcatt

SEQ ID NO: 29 - RNA, 21 nt, synthetic construct
  source 1..21: mol_type = other RNA
  modified_base 20..21: mod_base = OTHER; note = Thymine
tgcaatgagacagacagactt

SEQ ID NO: 30 - RNA, 21 nt, synthetic construct
  source 1..21: mol_type = other RNA
  modified_base 20..21: mod_base = OTHER; note = Thymine
gctggagaaagatcaaacatt

SEQ ID NO: 31 - RNA, 21 nt, synthetic construct
  source 1..21: mol_type = other RNA
  modified_base 20..21: mod_base = OTHER; note = Thymine
tgtttgatctttctccagctt

SEQ ID NO: 32 - RNA, 21 nt, synthetic construct
  source 1..21: mol_type = other RNA
  modified_base 20..21: mod_base = OTHER; note = Thymine
gcagctgacagacaccaaatt

SEQ ID NO: 33 - RNA, 21 nt, synthetic construct
  source 1..21: mol_type = other RNA
  modified_base 20..21: mod_base = OTHER; note = Thymine
tttggtgtctgtcagctgctt

SEQ ID NO: 34 - RNA, 21 nt, synthetic construct
  source 1..21: mol_type = other RNA
  modified_base 20..21: mod_base = OTHER; note = Thymine
ggtgcacagtttcaccgaatt

SEQ ID NO: 35 - RNA, 21 nt, synthetic construct
  source 1..21: mol_type = other RNA
  modified_base 20..21: mod_base = OTHER; note = Thymine
ttcggtgaaactgtgcacctt

SEQ ID NO: 36 - RNA, 21 nt, synthetic construct
  source 1..21: mol_type = other RNA
  modified_base 20..21: mod_base = OTHER; note = Thymine
agaccactgtgcagccttatt

SEQ ID NO: 37 - RNA, 21 nt, synthetic construct
  source 1..21: mol_type = other RNA
  modified_base 20..21: mod_base = OTHER; note = Thymine
taaggctgcacagtggtcttt

SEQ ID NO: 38 - RNA, 21 nt, synthetic construct
  source 1..21: mol_type = other RNA
  modified_base 20..21: mod_base = OTHER; note = Thymine
agatgtcagcactgtgttatt

SEQ ID NO: 39 - RNA, 21 nt, synthetic construct
  source 1..21: mol_type = other RNA
  modified_base 20..21: mod_base = OTHER; note = Thymine
taacacagtgctgacatcttt

SEQ ID NO: 40 - RNA, 21 nt, synthetic construct
  source 1..21: mol_type = other RNA
  modified_base 20..21: mod_base = OTHER; note = Thymine
gctttcgtgtgctggagaatt

SEQ ID NO: 41 - RNA, 21 nt, synthetic construct
  source 1..21: mol_type = other RNA
  modified_base 20..21: mod_base = OTHER; note = Thymine
ttctccagcacacgaaagctt

SEQ ID NO: 42 - RNA, 21 nt, synthetic construct
  source 1..21: mol_type = other RNA
  modified_base 20..21: mod_base = OTHER; note = Thymine
agaagatgatggacaagaatt

SEQ ID NO: 43 - RNA, 21 nt, synthetic construct
  source 1..21: mol_type = other RNA
  modified_base 20..21: mod_base = OTHER; note = Thymine
ttcttgtccatcatcttcttt

SEQ ID NO: 44 - RNA, 21 nt, synthetic construct
  source 1..21: mol_type = other RNA
  modified_base 20..21: mod_base = OTHER; note = Thymine
agatgatggacaagaaatatt

SEQ ID NO: 45 - RNA, 21 nt, synthetic construct
  source 1..21: mol_type = other RNA
  modified_base 20..21: mod_base = OTHER; note = Thymine
tatttcttgtccatcatcttt

SEQ ID NO: 46 - RNA, 21 nt, synthetic construct
  source 1..21: mol_type = other RNA
  modified_base 20..21: mod_base = OTHER; note = Thymine
caatggacatgattcccaatt

SEQ ID NO: 47 - RNA, 21 nt, synthetic construct
  source 1..21: mol_type = other RNA
  modified_base 20..21: mod_base = OTHER; note = Thymine
ttgggaatcatgtccattgtt

SEQ ID NO: 48 - RNA, 21 nt, synthetic construct
  source 1..21: mol_type = other RNA
  modified_base 20..21: mod_base = OTHER; note = Thymine
ggacatgattcccaagtcatt

SEQ ID NO: 49 - RNA, 21 nt, synthetic construct
  source 1..21: mol_type = other RNA
  modified_base 20..21: mod_base = OTHER; note = Thymine
tgacttgggaatcatgtcctt

SEQ ID NO: 50 - RNA, 21 nt, synthetic construct
  source 1..21: mol_type = other RNA
  modified_base 20..21: mod_base = OTHER; note = Thymine
ccttagttctctaagtcattt

SEQ ID NO: 51 - RNA, 21 nt, synthetic construct
  source 1..21: mol_type = other RNA
  modified_base 20..21: mod_base = OTHER; note = Thymine
atgacttagagaactaaggtt

SEQ ID NO: 52 - RNA, 21 nt, synthetic construct
  source 1..21: mol_type = other RNA
  modified_base 20..21: mod_base = OTHER; note = Thymine
gatgcaatattcagactgatt

SEQ ID NO: 53 - RNA, 21 nt, synthetic construct
  source 1..21: mol_type = other RNA
  modified_base 20..21: mod_base = OTHER; note = Thymine
tcagtctgaatattgcatctt

SEQ ID NO: 54 - RNA, 21 nt, synthetic construct
  source 1..21: mol_type = other RNA
  modified_base 20..21: mod_base = OTHER; note = Thymine
ccttcctcctcttgctctatt

SEQ ID NO: 55 - RNA, 21 nt, synthetic construct
  source 1..21: mol_type = other RNA
  modified_base 20..21: mod_base = OTHER; note = Thymine
tagagcaagaggaggaaggtt

SEQ ID NO: 56 - RNA, 21 nt, synthetic construct
  source 1..21: mol_type = other RNA
  modified_base 20..21: mod_base = OTHER; note = Thymine
ccattcagttgatgtttattt

SEQ ID NO: 57 - RNA, 21 nt, synthetic construct
  source 1..21: mol_type = other RNA
  modified_base 20..21: mod_base = OTHER; note = Thymine
ataaacatcaactgaatggtt

SEQ ID NO: 58 - RNA, 21 nt, synthetic construct
  source 1..21: mol_type = other RNA
  modified_base 20..21: mod_base = OTHER; note = Thymine
gttgatgtttattgagcaatt

SEQ ID NO: 59 - RNA, 21 nt, synthetic construct
  source 1..21: mol_type = other RNA
  modified_base 20..21: mod_base = OTHER; note = Thymine
ttgctcaataaacatcaactt

SEQ ID NO: 60 - RNA, 21 nt, synthetic construct
  source 1..21: mol_type = other RNA
  modified_base 20..21: mod_base = OTHER; note = Thymine
gatgtttattgagcaactatt

SEQ ID NO: 61 - RNA, 21 nt, synthetic construct
  source 1..21: mol_type = other RNA
  modified_base 20..21: mod_base = OTHER; note = Thymine
tagttgctcaataaacatctt

SEQ ID NO: 62 - RNA, 21 nt, synthetic construct
  source 1..21: mol_type = other RNA
  modified_base 20..21: mod_base = OTHER; note = Thymine
gataaagttcctccctcaatt

SEQ ID NO: 63 - RNA, 21 nt, synthetic construct
  source 1..21: mol_type = other RNA
  modified_base 20..21: mod_base = OTHER; note = Thymine
ttgagggaggaactttatctt

SEQ ID NO: 64 - RNA, 21 nt, synthetic construct
  source 1..21: mol_type = other RNA
  modified_base 20..21: mod_base = OTHER; note = Thymine
gctgggagacagacaactatt

SEQ ID NO: 65 - RNA, 21 nt, synthetic construct
  source 1..21: mol_type = other RNA
  modified_base 20..21: mod_base = OTHER; note = Thymine
tagttgtctgtctcccagctt

SEQ ID NO: 66 - RNA, 21 nt, synthetic construct
  source 1..21: mol_type = other RNA
  modified_base 20..21: mod_base = OTHER; note = Thymine
ggagacagacaactaactatt

SEQ ID NO: 67 - RNA, 21 nt, synthetic construct
  source 1..21: mol_type = other RNA
  modified_base 20..21: mod_base = OTHER; note = Thymine
tagttagttgtctgtctcctt

SEQ ID NO: 68 - RNA, 21 nt, synthetic construct
  source 1..21: mol_type = other RNA
  modified_base 20..21: mod_base = OTHER; note = Thymine
agacagacaactaactacatt

SEQ ID NO: 69 - RNA, 21 nt, synthetic construct
  source 1..21: mol_type = other RNA
  modified_base 20..21: mod_base = OTHER; note = Thymine
tgtagttagttgtctgtcttt

SEQ ID NO: 70 - RNA, 21 nt, synthetic construct
  source 1..21: mol_type = other RNA
  modified_base 20..21: mod_base = OTHER; note = Thymine
gctcaaggcttcctggatatt

SEQ ID NO: 71 - RNA, 21 nt, synthetic construct
  source 1..21: mol_type = other RNA
  modified_base 20..21: mod_base = OTHER; note = Thymine
tatccaggaagccttgagctt

SEQ ID NO: 72 - RNA, 21 nt, synthetic construct
  source 1..21: mol_type = other RNA
  modified_base 20..21: mod_base = OTHER; note = Thymine
ggtagagtgagacttcagatt

SEQ ID NO: 73 - RNA, 21 nt, synthetic construct
  source 1..21: mol_type = other RNA
  modified_base 20..21: mod_base = OTHER; note = Thymine
tctgaagtctcactctacctt

SEQ ID NO: 74 - RNA, 21 nt, synthetic construct
  source 1..21: mol_type = other RNA
  modified_base 20..21: mod_base = OTHER; note = Thymine
gtgaggacttctaatttaatt

SEQ ID NO: 75 - RNA, 21 nt, synthetic construct
  source 1..21: mol_type = other RNA
  modified_base 20..21: mod_base = OTHER; note = Thymine
ttaaattagaagtcctcactt

SEQ ID NO: 76 - DNA, 20 bp, synthetic construct
  source 1..20: mol_type = other DNA
tctgacttcaacagcgacac

SEQ ID NO: 77 - DNA, 20 bp, synthetic construct
  source 1..20: mol_type = other DNA
gccaaattcgttgtcatacc

SEQ ID NO: 78 - DNA, 22 bp, synthetic construct
  source 1..22: mol_type = other DNA
gtgtgctggagaaagatcaaac

SEQ ID NO: 79 - DNA, 21 bp, synthetic construct
  source 1..21: mol_type = other DNA
tggtcaggctatttcttgtcc

SEQ ID NO: 80 - RNA, 21 nt, synthetic construct
  source 1..21: mol_type = other RNA
  modified_base 20..21: mod_base = OTHER; note = Thymine
  modified_base 2: mod_base = OTHER; note = 2-O-methyl
  modified_base 5: mod_base = OTHER; note = 2-O-methyl
  modified_base 6: mod_base = OTHER; note = 2-O-methyl
  modified_base 9: mod_base = OTHER; note = 2-O-methyl
  modified_base 13: mod_base = OTHER; note = 2-O-methyl
  modified_base 15..16: mod_base = OTHER; note = 2-O-methyl
gcagctgacagacaccaaatt

SEQ ID NO: 81 - RNA, 21 nt, synthetic construct
  source 1..21: mol_type = other RNA
  modified_base 20..21: mod_base = OTHER; note = Thymine
  modified_base 1..3: mod_base = OTHER; note = 2-O-methyl
  modified_base 6: mod_base = OTHER; note = 2-O-methyl
  modified_base 8..10: mod_base = OTHER; note = 2-O-methyl
  modified_base 12..13: mod_base = OTHER; note = 2-O-methyl
  modified_base 16..17: mod_base = OTHER; note = 2-O-methyl
  modified_base 19: mod_base = OTHER; note = 2-O-methyl
tttggtgtctgtcagctgctt

SEQ ID NO: 82 - RNA, 21 nt, synthetic construct
  source 1..21: mol_type = other RNA
  modified_base 1..9: mod_base = OTHER; note = 2-O-methyl
  modified_base 10..12: mod_base = OTHER; note = 2-deoxy-2-fluoro
  modified_base 13..19: mod_base = OTHER; note = 2-O-methyl
  modified_base 20..21: mod_base = OTHER; note = Thymine
gcagctgacagacaccaaatt

SEQ ID NO: 83 - RNA, 21 nt, synthetic construct
  source 1..21: mol_type = other RNA
  modified_base 20..21: mod_base = OTHER; note = Thymine
  modified_base 1..19: mod_base = OTHER; note = 2-O-methyl
tttggtgtctgtcagctgctt

SEQ ID NO: 84 - RNA, 21 nt, synthetic construct
  source 1..21: mol_type = other RNA
  modified_base 20..21: mod_base = OTHER; note = Thymine
  modified_base 1..9: mod_base = OTHER; note = 2-O-methyl
  modified_base 10..12: mod_base = OTHER; note = 2-deoxy-2-fluoro
  modified_base 13..19: mod_base = OTHER; note = 2-O-methyl
  modified_base 1^2: mod_base = OTHER; note = Phosphorothioate
  modified_base 2^3: mod_base = OTHER; note = Phosphorothioate
gcagctgacagacaccaaatt

SEQ ID NO: 85 - RNA, 21 nt, synthetic construct
  source 1..21: mol_type = other RNA
  modified_base 20..21: mod_base = OTHER; note = Thymine
  modified_base 1..19: mod_base = OTHER; note = 2-O-methyl
  modified_base 1^2: mod_base = OTHER; note = Phosphorothioate
  modified_base 2^3: mod_base = OTHER; note = Phosphorothioate
  modified_base 17^18: mod_base = OTHER; note = Phosphorothioate
  modified_base 18^19: mod_base = OTHER; note = Phosphorothioate
tttggtgtctgtcagctgctt

SEQ ID NO: 86 - RNA, 21 nt, synthetic construct
  source 1..21: mol_type = other RNA
  modified_base 20..21: mod_base = OTHER; note = Thymine
  modified_base 6: mod_base = p
gcagcngacagacaccaaatt

SEQ ID NO: 87 - RNA, 21 nt, synthetic construct
  source 1..21: mol_type = other RNA
  modified_base 20..21: mod_base = OTHER; note = Thymine
  modified_base 1..3: mod_base = p
  modified_base 6: mod_base = p
  modified_base 8: mod_base = p
  modified_base 10: mod_base = p
  modified_base 12: mod_base = p
  modified_base 17: mod_base = p
nnnggngncngncagcngctt

SEQ ID NO: 88 - RNA, 21 nt, synthetic construct
  source 1..21: mol_type = other RNA
  modified_base 20..21: mod_base = OTHER; note = Thymine
  modified_base 1..3: mod_base = OTHER; note = 2-O-methyl
  modified_base 4: mod_base = OTHER; note = 2-deoxy-2-fluoro
  modified_base 5: mod_base = OTHER; note = 2-O-methyl
  modified_base 6: mod_base = OTHER; note = 2-deoxy-2-fluoro
  modified_base 7: mod_base = OTHER; note = 2-O-methyl
  modified_base 8: mod_base = OTHER; note = 2-deoxy-2-fluoro
  modified_base 9: mod_base = OTHER; note = 2-O-methyl
  modified_base 10..12: mod_base = OTHER; note = 2-deoxy-2-fluoro
  modified_base 13: mod_base = OTHER; note = 2-O-methyl
  modified_base 14: mod_base = OTHER; note = 2-deoxy-2-fluoro
  modified_base 15: mod_base = OTHER; note = 2-O-methyl
  modified_base 16: mod_base = OTHER; note = 2-deoxy-2-fluoro
  modified_base 17..19: mod_base = OTHER; note = 2-O-methyl
gcagctgacagacaccaaatt

SEQ ID NO: 89 - RNA, 21 nt, synthetic construct
  source 1..21: mol_type = other RNA
  modified_base 20..21: mod_base = OTHER; note = Thymine
  modified_base 1..3: mod_base = OTHER; note = 2-deoxy-2-fluoro
  modified_base 4: mod_base = OTHER; note = 2-O-methyl
  modified_base 5: mod_base = OTHER; note = 2-deoxy-2-fluoro
  modified_base 6: mod_base = OTHER; note = 2-O-methyl
  modified_base 7: mod_base = OTHER; note = 2-deoxy-2-fluoro
  modified_base 8: mod_base = OTHER; note = 2-O-methyl
  modified_base 9: mod_base = OTHER; note = 2-deoxy-2-fluoro
  modified_base 10..12: mod_base = OTHER; note = 2-O-methyl
  modified_base 13: mod_base = OTHER; note = 2-deoxy-2-fluoro
  modified_base 14: mod_base = OTHER; note = 2-O-methyl
  modified_base 15: mod_base = OTHER; note = 2-deoxy-2-fluoro
  modified_base 16: mod_base = OTHER; note = 2-O-methyl
  modified_base 17..19: mod_base = OTHER; note = 2-deoxy-2-fluoro
tttggtgtctgtcagctgctt

SEQ ID NO: 90 - RNA, 21 nt, synthetic construct
  source 1..21: mol_type = other RNA
  modified_base 20..21: mod_base = OTHER; note = Thymine
  modified_base 1..3: mod_base = OTHER; note = 2-O-methyl
  modified_base 1^2: mod_base = OTHER; note = Phosphorothioate
  modified_base 2^3: mod_base = OTHER; note = Phosphorothioate
  modified_base 4: mod_base = OTHER; note = 2-deoxy-2-fluoro
  modified_base 5: mod_base = OTHER; note = 2-O-methyl
  modified_base 6: mod_base = OTHER; note = 2-deoxy-2-fluoro
  modified_base 7: mod_base = OTHER; note = 2-O-methyl
  modified_base 8: mod_base = OTHER; note = 2-deoxy-2-fluoro
  modified_base 9: mod_base = OTHER; note = 2-O-methyl
  modified_base 10..12: mod_base = OTHER; note = 2-deoxy-2-fluoro
  modified_base 13: mod_base = OTHER; note = 2-O-methyl
  modified_base 14: mod_base = OTHER; note = 2-deoxy-2-fluoro
  modified_base 15: mod_base = OTHER; note = 2-O-methyl
  modified_base 16: mod_base = OTHER; note = 2-deoxy-2-fluoro
  modified_base 17..19: mod_base = OTHER; note = 2-O-methyl
gcagctgacagacaccaaatt

SEQ ID NO: 91 - RNA, 21 nt, synthetic construct
  source 1..21: mol_type = other RNA
  modified_base 20..21: mod_base = OTHER; note = Thymine
  modified_base 1..3: mod_base = OTHER; note = 2-deoxy-2-fluoro
  modified_base 1^2: mod_base = OTHER; note = Phosphorothioate
  modified_base 2^3: mod_base = OTHER; note = Phosphorothioate
  modified_base 4: mod_base = OTHER; note = 2-O-methyl
  modified_base 5: mod_base = OTHER; note = 2-deoxy-2-fluoro
  modified_base 6: mod_base = OTHER; note = 2-O-methyl
  modified_base 7: mod_base = OTHER; note = 2-deoxy-2-fluoro
  modified_base 8: mod_base = OTHER; note = 2-O-methyl
  modified_base 9: mod_base = OTHER; note = 2-deoxy-2-fluoro
  modified_base 10..12: mod_base = OTHER; note = 2-O-methyl
  modified_base 13: mod_base = OTHER; note = 2-deoxy-2-fluoro
  modified_base 14: mod_base = OTHER; note = 2-O-methyl
  modified_base 15: mod_base = OTHER; note = 2-deoxy-2-fluoro
  modified_base 16: mod_base = OTHER; note = 2-O-methyl
  modified_base 17..19: mod_base = OTHER; note = 2-deoxy-2-fluoro
  modified_base 17^18: mod_base = OTHER; note = Phosphorothioate
  modified_base 18^19: mod_base = OTHER; note = Phosphorothioate
tttggtgtctgtcagctgctt